European Patent Application EP 4 549 460 A1, published May 7, 2025. Title: 固定化的内切糖苷酶融合蛋白及其应用. Applicant: 启德医药科技（苏州）有限公司. The sequence listing filed with the application follows.

SEQUENCE LISTING (7 sequences)

SEQ ID NO: 1 - protein, 1160 aa, synthetic construct
  REGION 1..1160: note = Halo-Endo S2-His
MAEIGTGFPFDPHYVEVLGERMHYVDVGPRDGTPVLFLHGNPTSSYVWRNIIPHVAPTHRCIAPDLIGMGKSDKPDLGYFFDDHVRFMDAFIEALGLEEVVLVIHDWGSALGFHWAKRNPERVKGIAFMEFIRPIPTWDEWPEFARETFQAFRTTDVGRKLIIDQNVFIEGTLPMGVVRPLTEVEMDHYREPFLNPVDREPLWRFPNELPIAGEPANIVALVEEYMDWLHQSPVPKLLFWGTPGVLIPPAEAARLAKSLPNCKAVDIGPGLNLLQEDNPDLIGSEIARWLSTLEISGGGGGSGGGGSMDKHLLVKRTLGCVCAATLMGAALATHHDSLNTVKAEEKTVQTGKTDQQVGAKLVQEIREGKRGPLYAGYFRTWHDRASTGIDGKQQHPENTMAEVPKEVDILFVFHDHTASDSPFWSELKDSYVHKLHQQGTALVQTIGVNELNGRTGLSKDYPDTPEGNKALAAAIVKAFVTDRGVDGLDIDIEHEFTNKRTPEEDARALNVFKEIAQLIGKNGSDKSKLLIMDTTLSVENNPIFKGIAEDLDYLLRQYYGSQGGEAEVDTINSDWNQYQNYIDASQFMIGFSFFEESASKGNLWFDVNEYDPNNPEKGKDIEGTRAKKYAEWQPSTGGLKAGIFSYAIDRDGVAHVPSTYKNRTSTNLQRHEVDNISHTDYTVSRKLKTLMTEDKRYDVIDQKDIPDPALREQIIQQVGQYKGDLERYNKTLVLTGDKIQNLKGLEKLSKLQKLELRQLSNVKEITPELLPESMKKDAELVMVGMTGLEKLNLSGLNRQTLDGIDVNSITHLTSFDISHNSLDLSEKSEDRKLLMTLMEQVSNHQKITVKNTAFENQKPKGYYPQTYDTKEGHYDVDNAEHDILTDFVFGTVTKRNTFIGDEEAFAIYKEGAVDGRQYVSKDYTYEAFRKDYKGYKVHLTASNLGETVTSKVTATTDETYLVDVSDGEKVVHHMKLNIGSGAIMMENLAKGAKVIGTSGDFEQAKKIFDGEKSDRFFTWGQTNWIAFDLGEINLAKEWRLFNAETNTEIKTDSSLNVAKGRLQILKDTTIDLEKMDIKNRKEYLSNDENWTDVAQMDDAKAIFNSKLSNVLSRYWRFCVDGGASSYYPQYTELQILGQRLSNDVANTLKDHHHHHHHHHH

SEQ ID NO: 2 - protein, 222 aa, synthetic construct
  REGION 1..222: note = mAb-1 Light chain
DIQMTQSPSSLSASVGDRVTITCRASQDVNTAVAWYQQKPGKAPKLLIYSASFLYSGVPSRFSGSRSGTDFTLTISSLQPEDFATYYCQQHYTTPPTFGQGTKVEIKRTVAAPSVFIFPPSDEQLKSGTASVVCLLNNFYPREAKVQWKVDNALQSGNSQESVTEQDSKDSTYSLSSTLTLSKADYEKHKVYACEVTHQGLSSPVTKSFNRGECGALPETGG

SEQ ID NO: 3 - protein, 450 aa, synthetic construct
  REGION 1..450: note = mAb-1 Heavy chain
EVQLVESGGGLVQPGGSLRLSCAASGFNIKDTYIHWVRQAPGKGLEWVARIYPTNGYTRYADSVKGRFTISADTSKNTAYLQMNSLRAEDTAVYYCSRWGGDGFYAMDYWGQGTLVTVSSASTKGPSVFPLAPSSKSTSGGTAALGCLVKDYFPEPVTVSWNSGALTSGVHTFPAVLQSSGLYSLSSVVTVPSSSLGTQTYICNVNHKPSNTKVDKKVEPKSCDKTHTCPPCPAPELLGGPSVFLFPPKPKDTLMISRTPEVTCVVVDVSHEDPEVKFNWYVDGVEVHNAKTKPREEQYNSTYRVVSVLTVLHQDWLNGKEYKCKVSNKALPAPIEKTISKAKGQPREPQVYTLPPSREEMTKNQVSLTCLVKGFYPSDIAVEWESNGQPENNYKTTPPVLDSDGSFFLYSKLTVDKSRWQQGNVFSCSVMHEALHNHYTQKSLSLSPGK

SEQ ID NO: 4 - protein, 222 aa, synthetic construct
  REGION 1..222: note = mAb-2 Light chain
DIQLTQSPSSLSASVGDRVSITCKASQDVSIAVAWYQQKPGKAPKLLIYSASYRYTGVPDRFSGSGSGTDFTLTISSLQPEDFAVYYCQQHYITPLTFGAGTKVEIKRTVAAPSVFIFPPSDEQLKSGTASVVCLLNNFYPREAKVQWKVDNALQSGNSQESVTEQDSKDSTYSLSSTLTLSKADYEKHKVYACEVTHQGLSSPVTKSFNRGECGALPETGG

SEQ ID NO: 5 - protein, 451 aa, synthetic construct
  REGION 1..451: note = mAb-2 Heavy chain
QVQLQQSGSELKKPGASVKVSCKASGYTFTNYGMNWVKQAPGQGLKWMGWINTYTGEPTYTDDFKGRFAFSLDTSVSTAYLQISSLKADDTAVYFCARGGFGSSYWYFDVWGQGSLVTVSSASTKGPSVFPLAPSSKSTSGGTAALGCLVKDYFPEPVTVSWNSGALTSGVHTFPAVLQSSGLYSLSSVVTVPSSSLGTQTYICNVNHKPSNTKVDKRVEPKSCDKTHTCPPCPAPELLGGPSVFLFPPKPKDTLMISRTPEVTCVVVDVSHEDPEVKFNWYVDGVEVHNAKTKPREEQYNSTYRVVSVLTVLHQDWLNGKEYKCKVSNKALPAPIEKTISKAKGQPREPQVYTLPPSREEMTKNQVSLTCLVKGFYPSDIAVEWESNGQPENNYKTTPPVLDSDGSFFLYSKLTVDKSRWQQGNVFSCSVMHEALHNHYTQKSLSLSPGK

SEQ ID NO: 6 - protein, 214 aa, synthetic construct
  REGION 1..214: note = mAb-3 Light chain
DIQMTQSPSSLSASVGDRVTITCRASQDVNTAVAWYQQKPGKAPKLLIYSASFLYSGVPSRFSGSRSGTDFTLTISSLQPEDFATYYCQQHYTTPPTFGQGTKVEIKRTVAAPSVFIFPPSDEQLKSGTASVVCLLNNFYPREAKVQWKVDNALQSGNSQESVTEQDSKDSTYSLSSTLTLSKADYEKHKVYACEVTHQGLSSPVTKSFNRGEC

SEQ ID NO: 7 - protein, 450 aa, synthetic construct; identical to SEQ ID NO: 3
  REGION 1..450: note = mAb-3 Heavy chain